European Patent Application EP 4 353 825 A1, published April 17, 2024. Title: MODIFIED PROMOTER SEQUENCES. Applicant: Technische Universität Graz. The sequence listing filed with the application follows.

SEQUENCE LISTING (32 sequences)

SEQ ID NO: 1 - DNA, 10 bp, synthetic construct
  source 1..10: mol_type = other DNA
atccttttag

SEQ ID NO: 2 - DNA, 10 bp, synthetic construct
  source 1..10: mol_type = other DNA
gataaccgtg

SEQ ID NO: 3 - DNA, 500 bp, Komagataella phaffii
  source 1..500: mol_type = genomic DNA
taatcgaactccgaatgcggttctcctgtaaccttaattgtagcatagatcacttaaataaactcatggcctgacatctgtacacgttcttattggtcttttagcaatcttgaagtctttctattgttccggtcggcattacctaataaattcgaatcgagattgctagtacctgatatcatatgaagtaatcatcacatgcaagttccatgataccctctactaatggaattgaacaaagtttaagcttctcgcacgagaccgaatccatactatgcacccctcaaagttgggattagtcaggaaagctgagcaattaacttccctcgattggcctggacttttcgcttagcctgccgcaatcggtaagtttcattatcccagcggggtgatagcctctgttgctcatcaggccaaaatcatatataagctgtagacccagcacttcaattacttgaaattcaccataacacttgctctagtcaagacttacaattaaa

SEQ ID NO: 4 - DNA, 352 bp, Komagataella phaffii
  source 1..352: mol_type = genomic DNA
cttcagtaagagaaggaagcttggtgacgatcacagctatgatgtaatagaaattgctaagcaattgtgaggtgtgatgtattttgcagagcaattgtgcggtacaacggggtgttattgtcttcacaaggcatttattgcgaatttcgtagttgaaagaatattttagcacagggtgcttgacccctattgttgctcgctaaaccatgattgctaaatgatgacatagcaatcactttactaagattgctataaggacacctttcttagtataaatggacactcttttcccctgctaaacttcttttatttttcacacttaaacagttacaaaacacaaacacaactagaa

SEQ ID NO: 5 - DNA, 500 bp, synthetic construct
  source 1..500: mol_type = other DNA; note = PCTA1 variant
atccttttagccgaatgcggttctcctgtaaccttaattgtagcatagatcacttaaataaactcatggcctgacatctgtacacgttcttattggtcttttagcaatcttgaagtctttctattgttccggtcggcattacctaataaattcgaatcgagattgctagtacctgatatcatatgaagtaatcatcacatgcaagttccatgataccctctactaatggaattgaacaaagtttaagcttctcgcacgagaccgaatccatactatgcacccctcaaagttgggattagtcaggaaagctgagcaattaacttccctcgattggcctggacttttcgcttagcctgccgcaatcggtaagtttcattatcccagcggggtgatagcctctgttgctcatcaggccaaaatcatatataagctgtagacccagcacttcaattacttgaaattcaccataacacttgctctagtcaagacttacaattaaa

SEQ ID NO: 6 - DNA, 500 bp, synthetic construct
  source 1..500: mol_type = other DNA; note = PCTA1 variant
taatcgaactccgaatgcggttctcctgtaaccttaattgtagcatagatcacttaaataaactcatggcctgacatctgtacacgttcttattggtcttttagcaatcttgaagtctttctattgttccgataaccgtgacctaataaattcgaatcgagattgctagtacctgatatcatatgaagtaatcatcacatgcaagttccatgataccctctactaatggaattgaacaaagtttaagcttctcgcacgagaccgaatccatactatgcacccctcaaagttgggattagtcaggaaagctgagcaattaacttccctcgattggcctggacttttcgcttagcctgccgcaatcggtaagtttcattatcccagcggggtgatagcctctgttgctcatcaggccaaaatcatatataagctgtagacccagcacttcaattacttgaaattcaccataacacttgctctagtcaagacttacaattaaa

SEQ ID NO: 7 - DNA, 500 bp, synthetic construct
  source 1..500: mol_type = other DNA; note = PCTA1 variant
taatcgaactccgaatgcggttctcctgtaaccttaattgtagcatagatcacttaaataaactcatggcctgacatctgtacacgttcttattggtcttttagcaatcttgaagtctttctattgttccggtcggcattacctaataaattcgaatcgagattgctagtacctgatatcatatgaagtaatcatcacatgcaagttccatgataccctctactaatggaattgaacaaagtttaagcttgataaccgtgaccgaatccatactatgcacccctcaaagttgggattagtcaggaaagctgagcaattaacttccctcgattggcctggacttttcgcttagcctgccgcaatcggtaagtttcattatcccagcggggtgatagcctctgttgctcatcaggccaaaatcatatataagctgtagacccagcacttcaattacttgaaattcaccataacacttgctctagtcaagacttacaattaaa

SEQ ID NO: 8 - DNA, 500 bp, synthetic construct
  source 1..500: mol_type = other DNA; note = PCTA1 variant
taatcgaactccgaatgcggttctcctgtaaccttaattgtagcatagatcacttaaataaactcatggcctgacatctgtacacgttcttattggtcttttagcaatcttgaagtctttctattgttccggtcggcattacctaataaattcgaatcgagattgctagtacctgatatcatatgaagtaatcatcacatgcaagttccatgataccctctactaatggaattgaacaaagtttaagcttctcgcacgagaccgaatccatactatgcacccctcaaagttgggattagtcaggaaagctgagcaattaacttccctcgattggcctggacttttcgcttagcctgccgcaatcggtaaggataaccgtgccagcggggtgatagcctctgttgctcatcaggccaaaatcatatataagctgtagacccagcacttcaattacttgaaattcaccataacacttgctctagtcaagacttacaattaaa

SEQ ID NO: 9 - DNA, 500 bp, synthetic construct
  source 1..500: mol_type = other DNA; note = PCTA1 variant
taatcgaactccgaatgcggttctcctgtaaccttaattgtagcatagatcacttaaataaactcatggcctgacatctgtacacgttcttattggtcttttagcaatcttgaagtctttctattgttccggtcggcattacctaataaattcgaatcgagattgctagtacctgatatcatatgaagtaatcatcacatgcaagttccatgataccctctactaatggaattgaacaaagtttaagcttctcgcacgagaccgaatccatactatgcacccctcaaagttgggattagtcaggaaagctgagcaattaacttccctcgattggcctggacttttcgcttagcctgccgcaatcggtaagtttcattatcccagcggggtgatagcctctgttgctcatcaggccaaaatcatatataagctgtagacccagcacttcaattacttgaaattcaccataagataaccgtgagtcaagacttacaattaaa

SEQ ID NO: 10 - DNA, 500 bp, synthetic construct
  source 1..500: mol_type = other DNA; note = PCTA1 variant
taatcgaactccgaatgcggttctcctgtaaccttaattgtagcatagatcacttaaataaactcatggcctgacatctgtacacgttcttattggtcttttagcaatcttgaagtctttctattgttccgataaccgtgacctaataaattcgaatcgagattgctagtacctgatatcatatgaagtaatcatcacatgcaagttccatgataccctctactaatggaattgaacaaagtttaagcttgataaccgtgaccgaatccatactatgcacccctcaaagttgggattagtcaggaaagctgagcaattaacttccctcgattggcctggacttttcgcttagcctgccgcaatcggtaagtttcattatcccagcggggtgatagcctctgataaccgtgaggccaaaatcatatataagctgtagacccagcacttcaattacttgaaattcaccataacacttgctctagtcaagacttacaattaaa

SEQ ID NO: 11 - DNA, 500 bp, synthetic construct
  source 1..500: mol_type = other DNA; note = PCTA1 variant
taatcgaactccgaatgcggttctcctgtaaccttaattgtagcatagatcacttaaataaactcatggcctgacatctgtacacgttcttattggtcttttagcaatcttgaagtctttctattgttccgataaccgtgacctaataaattcgaatcgagattgctagtacctgatatcatatgaagtaatcatcacatgcaagttccatgataccctctactaatggaattgaacaaagtttaagcttgataaccgtgaccgaatccatactatgcacccctcaaagttgggattagtcaggaaagctgagcaattaacttccctcgattggcctggacttttcgcttagcctgccgcaatcggtaagtttcattatcccagcggggtgatagcctctgttgctcatcaggccaaaatcatatataagctgtagacccagcacttcaattacttgaaattcaccataagataaccgtgagtcaagacttacaattaaa

SEQ ID NO: 12 - DNA, 500 bp, synthetic construct
  source 1..500: mol_type = other DNA; note = PCTA1 variant
atccttttagccgaatgcggttctcctgtaaccttaattgtagcatagatcacttaaataaactcatggcctgacatctgtacacgttcttattggtcttttagcaatcttgaagtctttctattgttccgataaccgtgacctaataaattcgaatcgagattgctagtacctgatatcatatgaagtaatcatcacatgcaagttccatgataccctctactaatggaattgaacaaagtttaagcttgataaccgtgaccgaatccatactatgcacccctcaaagttgggattagtcaggaaagctgagcaattaacttccctcgattggcctggacttttcgcttagcctgccgcaatcggtaagtttcattatcccagcggggtgatagcctctgttgctcatcaggccaaaatcatatataagctgtagacccagcacttcaattacttgaaattcaccataacacttgctctagtcaagacttacaattaaa

SEQ ID NO: 13 - DNA, 500 bp, synthetic construct
  source 1..500: mol_type = other DNA; note = PCTA1 variant
atccttttagccgaatgcggttctcctgtaaccttaattgtagcatagatcacttaaataaactcatggcctgacatctgtacacgttcttattggtcttttagcaatcttgaagtctttctattgttccgataaccgtgacctaataaattcgaatcgagattgctagtacctgatatcatatgaagtaatcatcacatgcaagttccatgataccctctactaatggaattgaacaaagtttaagcttgataaccgtgaccgaatccatactatgcacccctcaaagttgggattagtcaggaaagctgagcaattaacttccctcgattggcctggacttttcgcttagcctgccgcaatcggtaaggataaccgtgccagcggggtgatagcctctgttgctcatcaggccaaaatcatatataagctgtagacccagcacttcaattacttgaaattcaccataacacttgctctagtcaagacttacaattaaa

SEQ ID NO: 14 - DNA, 500 bp, synthetic construct
  source 1..500: mol_type = other DNA; note = PCTA1 variant
atccttttagccgaatgcggttctcctgtaaccttaattgtagcatagatcacttaaataaactcatggcctgacatctgtacacgttcttattggtcttttagcaatcttgaagtctttctattgttccgataaccgtgacctaataaattcgaatcgagattgctagtacctgatatcatatgaagtaatcatcacatgcaagttccatgataccctctactaatggaattgaacaaagtttaagcttgataaccgtgaccgaatccatactatgcacccctcaaagttgggattagtcaggaaagctgagcaattaacttccctcgattggcctggacttttcgcttagcctgccgcaatcggtaagtttcattatcccagcggggtgatagcctctgttgctcatcaggccaaaatcatatataagctgtagacccagcacttcaattacttgaaattcaccataagataaccgtgagtcaagacttacaattaaa

SEQ ID NO: 15 - DNA, 500 bp, synthetic construct
  source 1..500: mol_type = other DNA; note = PCTA1 variant
atccttttagccgaatgcggttctcctgtaaccttaattgtagcatagatcacttaaataaactcatggcctgacatctgtacacgttcttattggtcttttagcaatcttgaagtctttctattgttccgataaccgtgacctaataaattcgaatcgagattgctagtacctgatatcatatgaagtaatcatcacatgcaagttccatgataccctctactaatggaattgaacaaagtttaagcttgataaccgtgaccgaatccatactatgcacccctcaaagttgggattagtcaggaaagctgagcaattaacttccctcgattggcctggacttttcgcttagcctgccgcaatcggtaaggataaccgtgccagcggggtgatagcctctgataaccgtgaggccaaaatcatatataagctgtagacccagcacttcaattacttgaaattcaccataagataaccgtgagtcaagacttacaattaaa

SEQ ID NO: 16 - DNA, 352 bp, synthetic construct
  source 1..352: mol_type = other DNA; note = PDH variant
cttcagtaaggataaccgtgttggtgacgatcacagctatgatgtaatagaaattgctaagcaattgtgaggtgtgatgtattttgcagagcaattgtgcggtacaacggggtgttattgtcttcacaaggcatttattgcgaatttcgtagttgaaagaatattttagcacagggtgcttgacccctattgttgctcgctaaaccatgattgctaaatgatgacatagcaatcactttactaagattgctataaggacacctttcttagtataaatggacactcttttcccctgctaaacttcttttatttttcacacttaaacagttacaaaacacaaacacaactagaa

SEQ ID NO: 17 - DNA, 352 bp, synthetic construct
  source 1..352: mol_type = other DNA; note = PDH variant
cttcagtaagagaaggaagcttggtgacgatcacagctatgatgtaatagaaattgctaagcaattgtgaggtgtgatgtattttgcagagcaattgtgcggtacaacggggtgttattggataaccgtggcatttattgcgaatttcgtagttgaaagaatattttagcacagggtgcttgacccctattgttgctcgctaaaccatgattgctaaatgatgacatagcaatcactttactaagattgctataaggacacctttcttagtataaatggacactcttttcccctgctaaacttcttttatttttcacacttaaacagttacaaaacacaaacacaactagaa

SEQ ID NO: 18 - DNA, 352 bp, synthetic construct
  source 1..352: mol_type = other DNA; note = PDH variant
cttcagtaagagaaggaagcttggtgacgatcacagctatgatgtaatagaaattgctaagcaattgtgaggtgtgatgtattttgcagagcaattgtgcggtacaacggggtgttattgtcttcacaaggcatttattgcgaatttcgtagttgaaagagataaccgtgacagggtgcttgacccctattgttgctcgctaaaccatgattgctaaatgatgacatagcaatcactttactaagattgctataaggacacctttcttagtataaatggacactcttttcccctgctaaacttcttttatttttcacacttaaacagttacaaaacacaaacacaactagaa

SEQ ID NO: 19 - DNA, 352 bp, synthetic construct
  source 1..352: mol_type = other DNA; note = PDH variant
cttcagtaagagaaggaagcttggtgacgatcacagctatgatgtaatagaaattgctaagcaattgtgaggtgtgatgtattttgcagagcaattgtgcggtacaacggggtgttattgtcttcacaaggcatttattgcgaatttcgtagttgaaagaatattttagcgataaccgtgtgacccctattgttgctcgctaaaccatgattgctaaatgatgacatagcaatcactttactaagattgctataaggacacctttcttagtataaatggacactcttttcccctgctaaacttcttttatttttcacacttaaacagttacaaaacacaaacacaactagaa

SEQ ID NO: 20 - DNA, 352 bp, synthetic construct
  source 1..352: mol_type = other DNA; note = PDH variant
cttcagtaagagaaggaagcttggtgacgatcacagctatgatgtaatagaaattgctaagcaattgtgaggtgtgatgtattttgcagagcaattgtgcggtacaacggggtgttattgtcttcacaaggcatttattgcgaatttcgtagttgaaagagataaccgtggataaccgtgtgacccctattgttgctcgctaaaccatgattgctaaatgatgacatagcaatcactttactaagattgctataaggacacctttcttagtataaatggacactcttttcccctgctaaacttcttttatttttcacacttaaacagttacaaaacacaaacacaactagaa

SEQ ID NO: 21 - DNA, 352 bp, synthetic construct
  source 1..352: mol_type = other DNA; note = PDH variant
cttcagtaaggataaccgtgttggtgacgatcacagctatgatgtaatagaaattgctaagcaattgtgaggtgtgatgtattttgcagagcaattgtgcggtacaacggggtgttattgtcttcacaaggcatttattgcgaatttcgtagttgaaagagataaccgtggataaccgtgtgacccctattgttgctcgctaaaccatgattgctaaatgatgacatagcaatcactttactaagattgctataaggacacctttcttagtataaatggacactcttttcccctgctaaacttcttttatttttcacacttaaacagttacaaaacacaaacacaactagaa

SEQ ID NO: 22 - DNA, 352 bp, synthetic construct
  source 1..352: mol_type = other DNA; note = PDH variant
cttcagtaagagaaggaagcttggtgacgatcacagctatgatgtaatagaaattgctaagcaattgtgaggtgtgatgtattttgcagagcaattgtgcggtacaacggggtgttattgtcttcacaaggcatttattgcgaatttcgtagttgaaagaatattttagcacagggtaaatgacccctattgttgctcgctaaaccatgattgctaaatgatgacatagcaatcaaattactaagattgctataaggacacctttcttagtataaatggacactcttttcccctgctaaacttcttttatttttcacacttaaacagttacaaaacacaaacacaactaaaa

SEQ ID NO: 23 - DNA, 352 bp, synthetic construct
  source 1..352: mol_type = other DNA; note = PDH variant
cttcagtaagagaaggaagcttggtgacgatcacagaaatgatgtaatagaaattgctaagcaattgtgaggtgtgatgtattttgcagagcaattgtgcggaaaaacaaagtgttattgtcttcacaaggcatttattgcgaatttcgtagttgaaagaatattttagcacagggtaaatgacccctattgttgctcgctaaaccatgattgctaaatgatgacatagcaatcaaattactaagattgctataaggacacctttcttagtataaatggacactcttttcccctgctaaacttcttttatttttcacacttaaacagttacaaaacacaaacacaactaaaa

SEQ ID NO: 24 - DNA, 352 bp, synthetic construct
  source 1..352: mol_type = other DNA; note = PDH variant
cttcagtaagagaaggaagcttggtgacgatcacagctatgatgtaatagaaattgctaagcaattgtgaggtgtgatgtattttgcagagcaattgtgcggtacaacggggtgttattgtcttcacaaggcatttattgcgaatttcgtagttgaaagagataaccgtggataaccgtgtgacccctattgttgctcgctaaaccatgattgctaaatgatgacatagcaatcaaattactaagattgctataaggacacctttcttagtataaatggacactcttttcccctgctaaacttcttttatttttcacacttaaacagttacaaaacacaaacacaactaaaa

SEQ ID NO: 25 - DNA, 500 bp, synthetic construct
  source 1..500: mol_type = other DNA; note = PCTA1 variant
taatcgaactccgaatgcggttctcctgtaaccttaattgtagcatagatcacttaaataaactcatggcctgacatctgtacacgttcttattggtcttttagcaatcttgaagtctttctattgttccggtcggcattacctaataaattcgaatcgagattgctagtacctgatatcatatgaagtaatcatcacatgcaagttccatgataccctctactaatggaattgaacaaagtttaagcttctcgcacgagaccgaatccatactatgcacccctcaaagttgggattagtcaggaaagctgagcaattaacttccctcgattggcctggacttttcgcttagcctgccgcaatcggtaagtttcattatcccagcggggtgatagcctctgataaccgtgaggccaaaatcatatataagctgtagacccagcacttcaattacttgaaattcaccataacacttgctctagtcaagacttacaattaaa

SEQ ID NO: 26 - DNA, 485 bp, synthetic construct
  source 1..485: mol_type = other DNA; note = PCTA1 variant
tgcggttctcctgtaaccttaattgtagcatagatcacttaaataaactcatggcctgacatctgtacacgttcttattggtcttttagcaatcttgaagtctttctattgttccggtcggcattacctaataaattcgaatcgagattgctagtacctgatatcatatgaagtaatcatcacatgcaagttccatgataccctctactaatggaattgaacaaagtttaagcttctcgcacgagaccgaatccatactatgcacccctcaaagttgggattagtcaggaaagctgagcaattaacttccctcgattggcctggacttttcgcttagcctgccgcaatcggtaagtttcattatcccagcggggtgatagcctctgttgctcatcaggccaaaatcatatataagctgtagacccagcacttcaattacttgaaattcaccataacacttgctctagtcaagacttacaattaaa

SEQ ID NO: 27 - DNA, 487 bp, synthetic construct
  source 1..487: mol_type = other DNA; note = PCTA1 variant
taatcgaactccgaatgcggttctccttagcatagatcacttaaataaactcatggcctgacatctgtacacgttcttattggtcttttagcaatcttgaagtctttctattgttccggtcggcattacctaataaattcgaatcgagattgctagtacctgatatcatatgaagtaatcatcacatgcaagttccatgataccctctactaatggaattgaacaaagtttaagcttctcgcacgagaccgaatccatactatgcacccctcaaagttgggattagtcaggaaagctgagcaattaacttccctcgattggcctggacttttcgcttagcctgccgcaatcggtaagtttcattatcccagcggggtgatagcctctgttgctcatcaggccaaaatcatatataagctgtagacccagcacttcaattacttgaaattcaccataacacttgctctagtcaagacttacaattaaa

SEQ ID NO: 28 - DNA, 479 bp, synthetic construct
  source 1..479: mol_type = other DNA; note = PCTA1 variant
taatcgaactccgaatgcggttctcctgtaaccttaattgtagcatagatcacttaaataaactcatggcctgacatctgtacacgttcttattggtcttttagcaatcttgaagtctttctattgttccggtcggcattacctaataaattcgaatcgagattgctagtacctgatatcatatgaagtaatcatcacatgcaagttccatgataccctctactaatggaattgaacaaagtttaagcttctcgcacgagaccgaatccatactatgcacccctcaaagttgggattagtcaggaaagctgagcaattaacttccctcgattggcctggacttttcgcttagcctgccgcaatcggtaagtttcattatcccagcggggtgatagcctctgttgctcttcaggccaaaatcatatataagctgtagacccagcacttaacacttgctctagtcaagacttacaattaaa

SEQ ID NO: 29 - DNA, 483 bp, synthetic construct
  source 1..483: mol_type = other DNA; note = PCTA1 variant
taatcgaactccgaatgcggttctcctgtaaccttaattgtagcatagatcacttaaataaactcatggcctgacatctgtacacgtttagcaatcttgaagtctttctattgttccggtcggttacctaataaattcgaatcgagttgctagtacctgtatcatatgaagtaatcatcacatgcaagttccatgataccctctactaatggaattgaacaaagtttaagcttctcgcacgagaccgaatccatactatgcacccctcaaagttgggattagtcaggaaagctgagcaattaacttccctcgattggcctggacttttcgcttagcctgccgcaatcggtaagtttcattatcccagcggggtgatagcctctgttgctcatcaggccaaaatcatatataagctgtagacccagcacttcaattacttgaaattcaccataacacttgctctagtcaagacttacaattaaa

SEQ ID NO: 30 - DNA, 353 bp, synthetic construct
  source 1..353: mol_type = other DNA; note = PDH variant
cttcagtaagagaaggaagcttggtgacgatcacagctatgataaccgtgaaattgctaagcaattgtgaggtgtgatgtattttgcagagcaattgtgcggtacaacggggtgttattgtcttcacaaggcatttattgcgaatttcgtagttgaaagaatattttagcacagggtgcttgacccctattgttgctcgctaaaccatgattgctaaatgatgacatagcaatcactttactaagattgctataaggacacctttcttagtataaatggacactcttttcccctgctaaacttcttttatttttcacacttaaacagttacaaaacacaaacacaactagaab

SEQ ID NO: 31 - DNA, 352 bp, synthetic construct
  source 1..352: mol_type = other DNA; note = PDH variant
cttcagtaagagaaggaagcttggtgacgatcacagctatgatgtaatagaaattgctaagcaattgtgaggtgtgatgtattttgcagagcaattgtgcggtacaacggggtgttattgtcttcacaaggcatttattgcgaatttcgtagttgaaagaatattttagcacagggtaaatgacccctattgttgctcgctaaaccatgattgctaaatgatgacatagcaatcactttactaagattgctataaggacacctttcttagtataaatggacactcttttcccctgctaaacttcttttatttttcacacttaaacagttacaaaacacaaacacaactagaa

SEQ ID NO: 32 - DNA, 500 bp, synthetic construct
  source 1..500: mol_type = other DNA; note = PCTA1 variant
taatcgaactccgaatgcggttctcctgtaaccttaattgtagcatagatcacttaaataaactcatggcctgacatctgtacacgttcttattggtcttttagcaatcttgaagtctttctattgttccggtcggcattacctaataaattcgaatcgagattgctagtacctgatatcatatgaagtaatcatcacatgcaagttccatgataccctctactaatggaattgaacaaagtttaagcttctcgcacgagaccgaatccatactatgcacccctcaaagttgggattagtcaggaaagctgagcaattaacttccctcgattggcctggacttttcgcttagcctgccgcaatcggtaaggataaccgtgccagcggggtgatagcctctgataaccgtgaggccaaaatcatatataagctgtagacccagcacttcaattacttgaaattcaccataagataaccgtgagtcaagacttacaattaaa